European Patent Application EP 4 545 631 A1, published April 30, 2025. Title: IMMUNE CELLS EXPRESSING IMMUNE CHECKPOINT MODULATOR AND USES THEREOF. Applicant: HK inno.N Corporation. Application KR. The sequence listing filed with the application follows.

SEQUENCE LISTING (38 sequences)

SEQ ID NO: 1 - protein, 246 aa, Artificial Sequence
EVQLLESGGGLVQPGGSLRLSCAASGFTFSDYAMSWVRQAPGKGLEWVSVISHDGGSIYYADSVKGRFTISRDNSKNTLYLQMNSLRAEDTAVYYCAKGPRRIANAIFDYWGQGTLVTVSSGGGGSGGGGSGGGGSQFVLTQPPSVSAAPGQKVTISCSGSNSNIGNSYVSWYQQVPGAAPRLLIYGSTNRPSGVPDRFSGSKSGTSASLAITGLQAEDEADYYCQSYDSSLSGYVFGTGTKVTVL

SEQ ID NO: 2 - protein, 246 aa, Artificial Sequence
EVQLLESGGGLVQPGGSLRLSCAASGFTFSDYAMSWVRQAPGKGLEWVSVISHDGDRVYYADSVKGRFTISRDNSKNTLYLQMNSLRAEDTAVYYCAKGPRRIANAIFDYWGQGTLVTVSSGGGGSGGGGSGGGGSQLVLTQPPSVSGAPGQKVTISCSGSSSNIGHSYVSWYQQLPGTAPKLLIYGDNNRPSGVPDRFSGSKSGTSASLAITGLQAEDEADYYCQSYDSSLSGYVFGTGTKVTVL

SEQ ID NO: 3 - protein, 246 aa, Artificial Sequence
EVQLLESGGGLVQPGGSLRLSCAASGFTFSDYSMSWVRQAPGKGLEWVSAISPDRSLEYYADSVKGRFTISRDNSKNTLYLQMNSLRAEDTAVYYCAKGPRHLTNNIFDYWGQGTLVTVSSGGGGSGGGGSGGGGSQFVLTQPPSVSAAPGQKVTISCSGSSSNIGHSYVSWYQQLPGTAPKLLIYGNIHRPSGVPDRFSGSTSGTSASLAITGLQADDEADYYCGVWDSSLSAVVFGGGTKLTVL

SEQ ID NO: 4 - protein, 497 aa, Artificial Sequence
MEFGLSWLFLVAILKGVQCEVQLLESGGGLVQPGGSLRLSCAASGFTFSDYAMSWVRQAPGKGLEWVSVISHDGGSIYYADSVKGRFTISRDNSKNTLYLQMNSLRAEDTAVYYCAKGPRRIANAIFDYWGQGTLVTVSSGGGGSGGGGSGGGGSQFVLTQPPSVSAAPGQKVTISCSGSNSNIGNSYVSWYQQVPGAAPRLLIYGSTNRPSGVPDRFSGSKSGTSASLAITGLQAEDEADYYCQSYDSSLSGYVFGTGTKVTVLEPKSCDKTHTCPPCPAPELLGGPSVFLFPPKPKDTLMISRTPEVTCVVVDVSHEDPEVKFNWYVDGVEVHNAKTKPREEQYNSTYRVVSVLTVLHQDWLNGKEYKCKVSNKALPAPIEKTISKAKGQPREPQVYTLPPSREEMTKNQVSLTCLVKGFYPSDIAVEWESNGQPENNYKTTPPVLDSDGSFFLYSKLTVDKSRWQQGNVFSCSVMHEALHNHYTQKSLSLSPGK

SEQ ID NO: 5 - protein, 497 aa, Artificial Sequence
MEFGLSWLFLVAILKGVQCEVQLLESGGGLVQPGGSLRLSCAASGFTFSDYAMSWVRQAPGKGLEWVSVISHDGDRVYYADSVKGRFTISRDNSKNTLYLQMNSLRAEDTAVYYCAKGPRRIANAIFDYWGQGTLVTVSSGGGGSGGGGSGGGGSQLVLTQPPSVSGAPGQKVTISCSGSSSNIGHSYVSWYQQLPGTAPKLLIYGDNNRPSGVPDRFSGSKSGTSASLAITGLQAEDEADYYCQSYDSSLSGYVFGTGTKVTVLEPKSCDKTHTCPPCPAPELLGGPSVFLFPPKPKDTLMISRTPEVTCVVVDVSHEDPEVKFNWYVDGVEVHNAKTKPREEQYNSTYRVVSVLTVLHQDWLNGKEYKCKVSNKALPAPIEKTISKAKGQPREPQVYTLPPSREEMTKNQVSLTCLVKGFYPSDIAVEWESNGQPENNYKTTPPVLDSDGSFFLYSKLTVDKSRWQQGNVFSCSVMHEALHNHYTQKSLSLSPGK

SEQ ID NO: 6 - protein, 497 aa, Artificial Sequence
MEFGLSWLFLVAILKGVQCEVQLLESGGGLVQPGGSLRLSCAASGFTFSDYSMSWVRQAPGKGLEWVSAISPDRSLEYYADSVKGRFTISRDNSKNTLYLQMNSLRAEDTAVYYCAKGPRHLTNNIFDYWGQGTLVTVSSGGGGSGGGGSGGGGSQFVLTQPPSVSAAPGQKVTISCSGSSSNIGHSYVSWYQQLPGTAPKLLIYGNIHRPSGVPDRFSGSTSGTSASLAITGLQADDEADYYCGVWDSSLSAVVFGGGTKLTVLEPKSCDKTHTCPPCPAPELLGGPSVFLFPPKPKDTLMISRTPEVTCVVVDVSHEDPEVKFNWYVDGVEVHNAKTKPREEQYNSTYRVVSVLTVLHQDWLNGKEYKCKVSNKALPAPIEKTISKAKGQPREPQVYTLPPSREEMTKNQVSLTCLVKGFYPSDIAVEWESNGQPENNYKTTPPVLDSDGSFFLYSKLTVDKSRWQQGNVFSCSVMHEALHNHYTQKSLSLSPGK

SEQ ID NO: 7 - protein, 22 aa, Artificial Sequence
GSGATNFSLLKQAGDVEENPGP

SEQ ID NO: 8 - protein, 19 aa, Homo sapiens
MEFGLSWLFLVAILKGVQC

SEQ ID NO: 9 - protein, 22 aa, Mus musculus
MDMRAPAGIFGFLLVLFPGYRS

SEQ ID NO: 10 - protein, 18 aa, Homo sapiens
MKWVTFISLLFLFSSAYS

SEQ ID NO: 11 - protein, 19 aa, Homo sapiens
MTRLTVLALLAGLLASSRA

SEQ ID NO: 12 - protein, 21 aa, Homo sapiens
MALPVTALLLPLALLLHAARP

SEQ ID NO: 13 - protein, 15 aa, Artificial Sequence
GGGGSGGGGSGGGGS

SEQ ID NO: 14 - protein, 232 aa, Homo sapiens
EPKSCDKTHTCPPCPAPELLGGPSVFLFPPKPKDTLMISRTPEVTCVVVDVSHEDPEVKFNWYVDGVEVHNAKTKPREEQYNSTYRVVSVLTVLHQDWLNGKEYKCKVSNKALPAPIEKTISKAKGQPREPQVYTLPPSREEMTKNQVSLTCLVKGFYPSDIAVEWESNGQPENNYKTTPPVLDSDGSFFLYSKLTVDKSRWQQGNVFSCSVMHEALHNHYTQKSLSLSPGK

SEQ ID NO: 15 - protein, 121 aa, Artificial Sequence
EVQLLESGGGLVQPGGSLRLSCAASGFTFSDYAMSWVRQAPGKGLEWVSVISHDGGSIYYADSVKGRFTISRDNSKNTLYLQMNSLRAEDTAVYYCAKGPRRIANAIFDYWGQGTLVTVSS

SEQ ID NO: 16 - protein, 110 aa, Artificial Sequence
QFVLTQPPSVSAAPGQKVTISCSGSNSNIGNSYVSWYQQVPGAAPRLLIYGSTNRPSGVPDRFSGSKSGTSASLAITGLQAEDEADYYCQSYDSSLSGYVFGTGTKVTVL

SEQ ID NO: 17 - protein, 121 aa, Artificial Sequence
EVQLLESGGGLVQPGGSLRLSCAASGFTFSDYAMSWVRQAPGKGLEWVSVISHDGDRVYYADSVKGRFTISRDNSKNTLYLQMNSLRAEDTAVYYCAKGPRRIANAIFDYWGQGTLVTVSS

SEQ ID NO: 18 - protein, 110 aa, Artificial Sequence
QLVLTQPPSVSGAPGQKVTISCSGSSSNIGHSYVSWYQQLPGTAPKLLIYGDNNRPSGVPDRFSGSKSGTSASLAITGLQAEDEADYYCQSYDSSLSGYVFGTGTKVTVL

SEQ ID NO: 19 - protein, 121 aa, Artificial Sequence
EVQLLESGGGLVQPGGSLRLSCAASGFTFSDYSMSWVRQAPGKGLEWVSAISPDRSLEYYADSVKGRFTISRDNSKNTLYLQMNSLRAEDTAVYYCAKGPRHLTNNIFDYWGQGTLVTVSS

SEQ ID NO: 20 - protein, 110 aa, Artificial Sequence
QFVLTQPPSVSAAPGQKVTISCSGSSSNIGHSYVSWYQQLPGTAPKLLIYGNIHRPSGVPDRFSGSTSGTSASLAITGLQADDEADYYCGVWDSSLSAVVFGGGTKLTVL

SEQ ID NO: 21 - protein, 5 aa, Artificial Sequence
DYAMS

SEQ ID NO: 22 - protein, 17 aa, Artificial Sequence
VISHDGGSIYYADSVKG

SEQ ID NO: 23 - protein, 12 aa, Artificial Sequence
GPRRIANAIFDY

SEQ ID NO: 24 - protein, 13 aa, Artificial Sequence
SGSNSNIGNSYVS

SEQ ID NO: 25 - protein, 7 aa, Artificial Sequence
GSTNRPS

SEQ ID NO: 26 - protein, 11 aa, Artificial Sequence
QSYDSSLSGYV

SEQ ID NO: 27 - protein, 5 aa, Artificial Sequence
DYAMS

SEQ ID NO: 28 - protein, 17 aa, Artificial Sequence
VISHDGDRVYYADSVKG

SEQ ID NO: 29 - protein, 12 aa, Artificial Sequence
GPRRIANAIFDY

SEQ ID NO: 30 - protein, 13 aa, Artificial Sequence
SGSSSNIGHSYVS

SEQ ID NO: 31 - protein, 7 aa, Artificial Sequence
GDNNRPS

SEQ ID NO: 32 - protein, 11 aa, Artificial Sequence
QSYDSSLSGYV

SEQ ID NO: 33 - protein, 5 aa, Artificial Sequence
DYSMS

SEQ ID NO: 34 - protein, 17 aa, Artificial Sequence
AISPDRSLEYYADSVKG

SEQ ID NO: 35 - protein, 12 aa, Artificial Sequence
GPRHLTNNIFDY

SEQ ID NO: 36 - protein, 13 aa, Artificial Sequence
SGSSSNIGHSYVS

SEQ ID NO: 37 - protein, 7 aa, Artificial Sequence
GNIHRPS

SEQ ID NO: 38 - protein, 11 aa, Artificial Sequence
GVWDSSLSAVV